European Patent Specification EP 3 626 683 B1, published May 22, 2024. Title: A PROCESS FOR BIO-SLUDGE REDUCTION IN HYDROCARBON REFINERY EFFLUENT TREATMENT PLANT THROUGH MICROBIAL INTERVENTIONS. Applicant: Indian Oil Corporation Ltd. Application 201821033799. The sequence listing filed with the application follows.

SEQUENCE LISTING (15 sequences)

SEQ ID NO: 1 - DNA, 498 bp, DNA
tcaagcggaagcgataagcctttgccttccttgtttgataaagctttctttcattgaccatagatgataaaaatagtctgtctgctcgtccttgtcttttgctaaaaggtcgctgtactctgtttttgaaaagaagcgcttggcgatctcaaggctgatcggtttcgttttttcgatatctatgccgatcggctgtgaatcaaacgcgcaaatgacccagcgtccggagtgagaaatgttgaaatgagcgtcgggaagatcagggatgcacggcttcccgtattcctgcgtgctaaagcggatatcggatttgtccaactgatactgcctgcttatgactgagcgaacgagcacatctcccagcagggtgcggtgagcatcttctttatgataaaatctccggcatttctcccgtttttcaggtgatatgaaagacatgaaccgttcattttcttcctgtgaaagcgggcggtccatataaattccgtaaatcttcat

SEQ ID NO: 2 - DNA, 729 bp, DNA
atgagccaactcttcaaatcatttgatgcgtcggaaaaaacacagctcatctgttttccgtttgccggcggctattcggcgtcgtttcgccctctccatgcttttttgcagggggagtgcgagatgctcgctgccgagccgccgggacacggcacgaatcaaacgtcagccattgaggatctcgaagagctgacggatttgtacaagcaagaactgaaccttcgccctgatcggccgtttgtgctgttcggacacagtatgggcggaatgatcaccttcaggctggcgcaaaagcttgagcgtgaaggcatctttccgcaggcggttatcatttctgcaatccagccgcctcatattcagcggaagaaagtgtcccacctgcctgatgatcagtttctcgatcatattatccaattaggcggaatgcccgcagagcttgttgaaaataaggaggtcatgtcctttttcctgccttctttccgatcagattaccgggctcttgaacaatttgagctttacgatctggcccagatccagtcgcctgttcatgtctttaacgggcttgatgataaaaaatgcatacgagatgcggaagggtggaagaagtgggcaaaagacatcacattccatcaatttgacggcgggcacatgttcctgctgtcacaaacggaagaagtcgcagaacggatttttgcgatcttgaatcagcatccgatcattcaaccgtga

SEQ ID NO: 3 - DNA, 888 bp, DNA
tcaggcgtagccgatggccatctcgtggaatcccgccgcgcgttccgcccgctgcggctccggttgcttcagcaggtgctcgagcagggcgcggtgcacgcgtaccgctgccagcttggactccaggtcgaggaaatgcccggtgccctccacccgcgagaaactgcagtgcggcaggtagtcgcggaactggcgggcgtcctcggcggtggtgtattcgtcccagctgccgttgatgaaatgcacgtggctctggatccgctccaggcaagccaagtagccccgatcgttgagcgccagcacctggtcgatgtgaaagcgcgcctgctcgtattcgccggtggccagcgaagccatgtgctgatggttgctggctttcaggcgctgcggcaggtatttgccgacggtctcgttgagcagatggccgatcgccgacttgtcgtccagctcgatcagcgcctgcgcccgcccgacgtagtcgagcatcgcctggttcagtccaggggcgaatgccatcaccaccgagctgcggatgccgcgcggattgcgcgacagcgccagcagcgtggagataccgccccaggacgcggagaccaggtgattgacctcgaagcgctcgatcagcgccaggaggatttccacctcgtcgtccttggtgatcaacccgcgctgcgggttgtgctgacgcgactgcccggcgaagggcaggtcgaacagcaccacgttgaaatgttcggccaggcacttgcaggtccgggcgaacgaggcggtggtcgccatcgcgccgttgaccagcatcaccgtgctgcgcccgggatcctgcccaacgcgctcgacatgtacccgcaggcccttgcaaaccgataccaacagactttcgcgccgcat

SEQ ID NO: 4 - DNA, 978 bp, DNA
ctaggccttggccttgccggaagctacggacgccacggccgggccggcgaggcgcttcagcaggcgcgggcggttggtctccagcgcgccgccgcgtccccgcaggccgtcccacaggccccagcccaggcagcgcagcttgagcagcttgtcgcgttcgagcaggagcaccgcgaggccctgggtcagggtcggcaggttcgccagcagggccagcggcgaggaccgggcgtagcggcgcaggaccagcaggccgttgcgcgccaggtagtagcggcgcagcggggcgtggttcatcgcgctgaggctgagaccgccgaggcggcgggtcttgcgcgtgccgatgcggtgctcgaggaccagccgcgggtcgacgtacaggggcacgtccagcgcctgggcgcgcaggctgtattcggtgtccacgtggtcgatgaacagttcctcgtcgaagtggccgaggcgctggtaggcctcgcgggtcagcaggcagccggaggagatcaggaacgaggtgcgctgcggggtcgtcaggccgtccagagacaattgcctgagcgtcagtccgtcgagatggatggccggcaggaagcgccggtcaccccggtcgaagatccgtgggccgagcaggcaggcctgaccgttgcgcgcctgcaggttgcgccactgggcggcgaggaaggcgccgccgggacgggagtcctggtcgagcagcagcacaccctgcacgccacgccggaatagcgcgtcgagtccctggttgaaggcgccggcgatgccctgccggttgccgtggtgcagcacggcgatgccttgcccgcgcagccgggcattgcgctgcggatcgctgtgcggtgagttgtcgacggcaaggaagcgcagttgcggaaacgccgccgccagttcgccaaggtgttccaggtcgtcgtcgccaggattgaacagtaccaccagcacgcccatgtctatccggtccat

SEQ ID NO: 5 - DNA, 891 bp, DNA
atgaatactgattttgtgaagactcaacccgtccaaactcttctcgaccgcgccagcggcgtcgatgtggagggcggcgaccgtcggctcaaggccattacccgcgacctcgtcgaagcggtgatgacggtcatcgtcaagcatgacatcaacgaaagcgaattctggaaagcgatagactttttccagaagggcgccggtgaattcggcctgatcgtgccgggcgttggcctggaacatttccttgacctctacatggatgccaaggacgcggaagccgggctgtcgggcggcacgccgcgcaccattgaagggccgctctatgtcgcgggcgcgccgctggtcgaaggtgacgtcaacctttccgacgacgcggacgataccggcacgctgtacatgtccggcaccgtcaccggcccgaatggtgagcccgtcaccgatgccattctgcatgtctggcacgccaattcgatgggttggtattcgcatttcgaccccacgcgcgagcagacgccgttcaataaccgccgccggatcaagctcggcaaggacgggcgctattccttccattcgaagatgcccaatggctacagcgtgccccccggcggcgcgaccgatcagctgatgaaagccgtcggccgtcacggcaaccgtcctgcccacgtgcatttcttcgtagaagcgccgggctatcgcacgctgacgacgcagatcaatttcggtgacgatccgttcgcagccgacgactttgcgttcggcacccgcgaaggtctgctgccagtcccgaaccgtcagggcgacaccgtccatatcgcgttcgacttccagttgcagaagtctgctgaggcaacggatgaaagcttctccgctcgcagccgcttggccgtctga

SEQ ID NO: 6 - DNA, 933 bp, DNA
atgaccgtgaagatttcccagactgccgacatccagaagttcttcgaagaagccagtggcgccctgaatgaccagggcaacccgcgcgtgaagaacctcgtcctgcgaatcctgcaggacaccgcgaaactgatcgaagacatgaatgttacgcccgacgaattctggaaggcggtggactacctcaaccgccttggctcccgtcaggaggccggcctggtcgtcgccggcctcggcgtcgagcactacctcgacctgctgctggacgcccaggacgcggctgccggcctcggcggcggtaccccgcgcaccatcgaaggcccgctgtacgtggccggcgcgccgctgtccgaaggcgaagcgcggatggacgacggcaaggatgcgggcaccgtgatgtttctttccggccgcgtgttcgacccgcagggcaagccgctggccggcgcggtggtcgatctctggcacgccaacacccagggcacctactcgtacttcgacagcacccagtccgagttcaacctgcgccggcgcatcgtcaccgacgccgaagggcgctaccaggcgcgcagcatcgtgcccagtggctacggctgtccgccggatggcccgacccaggagttgctcgatcagctcggccgccacggccagcgcccggcgcacatccacttcttcatctccgcgccggggcatcgccacctgaccacgcagatcaacctcgccggcgaccagtacctgtgggacgacttcgcctacgccacccgcgacgggctgatcggcgaggtgcgtttcgtcgaagacgcagaggccgcgaaggtgcgcggtgtggaagggcgtttcgccgagatcgagttcgacttccagttgcagcaggcggtttccgctgatgccgaggaccgcagcaaccgtccccgcgcgctgcaggaagcctga

SEQ ID NO: 7 - DNA, 1464 bp, DNA
ctaggcctcctttgtgaggatttggtcggccgggatggcagtgctcccgacggcggcccgtgaaggatccgcctcggcggccgcgggtgcctgaataggatcggttccgacgtgcagctgggccgctttctccatcggtcggtcgaggtgatcagcccaccgcagcaggagttcacgctggttgtattcgctatagccgacccgcgtggaacctggtcctgaatactcatctgaggtcaggggttctacgacgttctgcccgttttccagcatgcccatccggctgttgagcaggaggcggcgggccatagggccgcccgccgtgctcgtcagcgagacccagttttcaacgtcgtcttgttcaaacatgccgccgctgccaaagcacatgagatatgccttgtacgaaagggccttgaactcctcagaggcgttcttgtccacggcaaaccacgaaacgatctcggtctcgtcttcgctgatgggctgccattggcggatggagataaacggcaggacttcgtcggagtcttcttctacgcggggccagttgtggacgaagctcatgtttgggaagaccgatgcggccgagaccatgaatccgtccttgcccacgacatcgagctgctcctggctccattgctccttcatccgcgcgatcatgtcgtcggggtagccgacatagcgaagccgttcctccaaggtgccctcgggaagcttgtaggtggtaccgccgccgttgccggcccagtaggttgttccatccttgcgcttctcagccttgggttcgcggaagagaccgatttcaacaactgacgtgtgcgtttggggagtgtggtacatgtcgccagcgaagttttcggcgccgatcttccagttcgctttgacccgccaccgctgggggccccggagttcgatgccgtcagcgctttgcttcgtgtagtaatccatgtagaacttgaagtcgcccaggaagtcctcgaggggttccgcgtcagggtcaaggctgatgaaaatcagcccgttgtaggtgcccaaggacggggcgggcagcagggtctgaccttttttcttgaagccctcttcgccgccgtaggcttctttgtggaacggcaggcccacgatgcgtccgtcgttgcggtaggaccagccgtggtaggggcagcggaaatgcgaggcgtttcccatctcggcccggcagacctgcatgccccggtggaggcacatgttaaagagagcacggatctcgcccttttcgtctcgggaaatgatgaatgaatcttcgagtactcggcgcactacgtagtcgccggcttcgggcacctcggactcgtgggcaacgaagagccaactccgtccgaagaggcgctccttttcgagctcgaagatttccttgtcgttgtaaatgtgtgcaggaatcatgccgcgctgcacgtcctggatgacgctggtctggtctgtcat

SEQ ID NO: 8 - DNA, 1290 bp, DNA
ttacttctcggcgaccaggcgggcgtgggcggattcctcgcccaggttgttcagcagccgctcgctgtaccagtcgaggaagttgatcacgccaaactcgtaggtcttggagtacggccccggctggtaggcggtggagttgatcccgcgctggttctcttcggccagccggcggtcctggtcgttggtggcgtcccacacttcgcgcaggcgcgccacgtcatagtcgacgccctccaccgcgtccttgtgcaccagccacttggtggtgaccacggtttcctgggcgctgatcggccacacggtgaagacgatcaggtggtcgcccatgcagtggttccacgagtgcggcaggtgcaggatgcgcatggagcccaggtccgggttcttgatgcgacccatcagcttcttcgagccctgcttgccgtccatcgtcatggacacggtgccgtcgagcagcggcatgcgcacgatgcggttgcgcaggccgaagctttcgtgggcgtaggggatcttctcctcgtcccaggccctggtgcaggcggcgacctgatccttgaacgcctgactggcgcgcgggtcggtgacatcgtcccactccagcagggtcttgagcagttcggggtgcgagccgttgcagtggtagcactcgcggttgttctcgagcaccagcttccagttggccgcttcgcggatcgtggtctgcaccgcgaccttggcgttctccatgtcgtacggctccatgtagtgctcgagcgtccgcaggaagtcgtcgatggccggcggattctccgccagcgaaatgaagatgtagccgccggcggtcttcacgttcaccggtttcaggctgtagtcctgcatgtcgaagtcggcgcccatttcggtgccggcgaacagcaggcggccgtccagttcgtaggtccactggtgataggggcagaccagcttggcgaccttgcccttgtcgctgacgcacaggcgcgagccacggtggcggcagacgttgtggaaggcgtggatctgcccttccgcgccgcgcaggacgatgaccgggttgtcgccgatctgcagggtgagaaagctgcccttggtcggaatctcgcaggtcatgccggcaatcagccactccttgtggaagatctcctgcatgtcgatctggaacaggcgctcgtcgttatagaagggctgcggcagcgagaagctgtggtcgcggctctgcagcatctcggcggtggccttgcgggccggctccagcggatcgcccagactcagggtagtggtgacgtccat

SEQ ID NO: 9 - DNA, 1167 bp, DNA
tcacggcgcgttcgcgatggcgagctccgcgagcaccttttgccggatcgacggcttgatgttcgattgcgccatgtccgcaccgtagtgcgcgacgacccgcggattcatcaccctgaaccacagcggcggcacgtacgcgagcaggatcatcgccgcgtagccggccggcagttgcggcgaatcgtcgaagtgccgcagcgcctgatacgagcgcgtcggattcgcatgatgatcggcgtggcgttgcaactgatagaggaacagattcgtcacgacgtggttgctattccacgagtgctgcggcgtgcagcgctcgtagcgtccggtcggcaactgcctgcggccgagcccgtaatgctcgacatagttcacgacctcgagcagcgacgcgccgtatgccgcctggatcagcaggaacggcaccaccttcgcgccgccgaacgcgatcgcggcgctccatagcgcgaccgtcatcgcccacgcctgcagcacctcgttgcgccacgaccacgccgagcggccgctgcgcgcgaggcgcgccttctcgagccgccatgcggacgcgatgctgcccgtcacggtgcgcggcaggaacgcccagaacgattcgccgtagcgcgcgctcgcgggatcgtccggcgtcgccacgcgcacgtggtgcccgcgattgtgctcgacgaagaagtggccgtacgcgacgggcgcgagcgtgatcttcgcgagccagcgctcgagcgggctcgtcttgtggccgagctcgtgcgcggtgttgatcgagatgccggtggccgcgccgagcgagaacgcgaagccgaggtagtcgtaccacgcgagcggctgcgtggcgacgatccagatcgcgcccgcgaaggcgacatagacgacgaaggtcgccagatagacgacgtagcggtagtagcgttcgctttcgagccggggcccgatcgattcgggcggattctcgctgtcgacgccgatcagcaggtcgagcaccgggatgacgccgaacgcgaagagcggcccgaaccaccagaacacgtgccagccggtcgacagcgcgaggagcgcggcgacgagcggcagcgtgatcgtcagtgcgccgagcagccaccaatagcgtttcgtgtcggcccagtcggccgacaccggttgctggattgccat

SEQ ID NO: 10 - DNA, 1149 bp, DNA
tcaggaagctgccggccgctcgctctgttcggccgtcaactggaactcttcgcccgcatagtaggcccgcaccttggggtccatgaccgcccgccacagcggcgggatcagcgccagcaccaccatcccggcataaccgctgggcatctgcgggctatcgtcataatgacggaggacctgataggggcgtttggcgaaggcatgatggtcggaatgccgttgcagatggaacaggaccaggttggtgaagacgaagttgctgttccaggagtgggtatggttggtccgctcgtagcgcccgtcctcgccctttcgccgatgcaggccgtagtgctcgacgtagttgatgatctccagcagggtcaccgcgacgaacgcttggccaaggaagaaaaccatccccagccagccgaacgcccaaccgaaaccgaccagcaacgccaggctcagcaggtaccaccagatcagttcgttctgccagccgaacaccggcaggcccttcttgcgcagccgcaccgcttcaaggcgccaggcgttgaggaagttgtacttgtaggcatgcggcaggaactggtagaccgactggccgaaacgcgccgacgaagcgtcctccggcgtagacacatgcacatggtggccgcgcacatgctcgaccttgaaccccgcgtagcacacggcggccagcaggatgccgccggcagcctgctccagcgccgagtccttgtggatcagctcatgggcgacgacgatccccaccgctcccatcaccgtgcccatcgagaggatccagcccaaccggccgagccagccccactcctggaaagcgacgaacacgccagcggcccacaccagcgtaccgatgagcaccggcaccgtggccagggtcagcaatacgtaatagccctggccgagcaactgcggcgtctgggtttcctcgtcggggttggccgggtcgcggccgaacagcatgtccagcagcggcccgatgccgaataccgcaatcaccagggaaaatgcccagaaggccggatgtgcgctgtcctgggccatccagtagttgaacggcatggacaacgccagcagcagccagagccaataggcgtacttcttgatggccagcatggtgctgggagagaaattttcaaacat

SEQ ID NO: 11 - DNA, 1224 bp, DNA
atgaatgcaccagtaaatgttcagcaagaacttatgccagtgccagcgtctatgcgtgagatagatcgtaagcgctatttatggatgattagtccggctctacctgtaattggtttaggtattttagctggataccattttggtccacgcccattaaagaaagtatttgctttaggtggcccacttttattacacgttgtgattcctgcaattgatacaattattggtaaagatgcgcgtaatccaaccgatgaagaaattaaacttcttgagaaagatccatattattcgcgtttggtaaaaagttttattccattgcagtatgcggcaaatatttatgcatgttatttaacaagccgtaaagatacttcatttattgacaaaattttgcttggtatttcgatgggtgccattaatggtattgcaattaatacagcccatgaattaagccataaacatgatcgtatagaccatattttatctcatcttgctctggtgcctacaggttacaaccatttccgtattgagcatccatatggccatcataagcgtgcagcgactcctgaagatccggcatcttcacgtatgggtgaaacattctatgaattttggccacgtactgttatcggttcttttaaatcagcaattgaaattgagaaaaatcgtttaaaacgtaaaggtaaagagttttggtcactcgataatgaattgctgcaaggctggggtatgagtgctgctttccatgcttctatggtaggaatttttggtaaaggtacgattccatatttggcaacacaagcattttacgggattagcctattcgaaattattaactatattgaacattatggcttattgcgtcagaaaaaaggaaatggccaatatgaacgtacaatgccagagcatagctggaataataacaatgtagtgaccaacttattcttatatcagttacagcgtcactcagatcatcatgcttatccaactcgtccattccaagcgttacgtcattttgatgaagcaccagagttgccaagtggctatgcaagtatgctgctaccagccatgattccttcatggtggtttaaaatgatggataagcgtgtatttgatcactacaaaggggatttaaataaagcaaatatttcaccaaaacgtcgtgcaaaaatcttcaaaaaatttggtgtagtcgataagtccttagaagctacacaggctgaataa

SEQ ID NO: 12 - DNA, 663 bp, DNA
atgtattcaggatcgcaatccggcggcaccgatcaggaacaaaacgtgtcgctgctggtggcgggcgatcacgaattgcttcgggatgccatcagcgaaatcctgagacgggagggagggttctcggtagaggtgaccggcagccgcgaaggggtgctcaagcagatcgaagaaagaggcgggttcgacgtcatcctgctcgatctgcagatgccgggcatgagcgggctcgattctctgcgcgaagtagcgacgtcaaatgccaacggagccgtagcgattttagcgggcgagcttacgcgcgatgtggtgatgagtgccttcaaggcaggcgccagaggctatattccgaaaacactcccgctgcgcgccttgcccatcgccttgcgcctcatcgcctccggtgagagttacgttcctgcgtggctgacaaatggaggcggaacaacgcaggcggatggccccagtttcgatcttctgccagaagagttgcagatcctggaagaggtttcggacgggcggaccaacaagcagatcgctttcacgctgaacgtgaccgaaggtgccatcaagatgaagatgcgcgccatctgcatgaagctgggagccaagaaccggacgcacgcggtggtgatcgcgcggcagcacatgatgctgcggtga

SEQ ID NO: 13 - DNA, 681 bp, DNA
atgggtaagcccttgccgcgcgatcagcttgctaaaaacgtcgcagccacggctgctgccggtaacgttgcaggcgcactggatctgctcgtaacctatgctggcgcctcgcattatttgctggcgcgagatgatcttctcgaagaaaccgggctgaaattcatcgtcacatccgactggcctttcgatctggtccgcaggctcggcattgaactcaccaacagccagaaccggtcgagcgaaatggagaagtgcctttcgctgcttcagccgcgattgcttctccttcccgacgatgtttccgtgccctatggcatagacaggcaatattcggcactctccttttgtgtgggccgcatccgcctttcccttttgctgctgtttccggaagaagcggttccgtcaccggagcgcctgcgggaaatcgccctgctgacggggtattgcgtcagcttcggcatcgccagcgaagcaaagaccgtgcgcgatatcgatctcaccgagcgtgagctcgagtgcctgttctggatcgcggaaggcaagacaagtgatgaaattgcgatgatccttggcatttcacgcaatacgatcaataattacatcacaagcgtgatgcgtaaaaccgcgacaaaaacccgctcggaggcaattgcctacgccgtgcgcaacaacctcgtataa

SEQ ID NO: 14 - DNA, 591 bp, DNA
atgatcaccgttgcccttatagacgatcacctcatcgtccgctccggctttgcgcagctgctggggctggaacctgatttgcaggtagttgccgagtttggttcggggcgcgaggcgctggcggggctgccggggcgcggtgtgcaggtgtgtatttgcgatatctccatgcccgatatctccggtctggagctgctaagccagctgccgaaaggtatggcgacgattatgctctccgttcacgacagtcctgcgctggttgagcaggcgcttaacgcgggggcacgcggctttctttccaaacgctgtagcccggatgaactcattgctgcggtgcatacggttgccacgggcggctgttatctgacgccggatattgccattaaactggcatccggtcgtcaggacccgctgaccaaacgtgaacgccaggtggcggaaaaactggcgcaaggaatggcggtgaaagagattgccgccgaactgggcttgtcaccgaaaacggtacacgtccatcgcgccaatctgatggaaaaactgggcgtcagtaacgacgtagagctggcgcgccgcatgtttgatggctggtga

SEQ ID NO: 15 - DNA, 531 bp, DNA
atgtttcttataattaccagggatacgatgttcttcaccgcgatgaaaaacattctgagtaaaggtaatgtcgttcatatacagaacgaagaagagatcgacgtaatgttgcatcagaatgccttcgtcattattgatacattaatgaataatgtatttcattctaattttctcactcaaattgaacgattaaaacctgtccatgtcattattttctccccctttaatattaaacgctgcctggggaaagtgccggtgacctttgttccgcggactatcactatcattgattttgtcgcactcatcaatggcagttactgctctgtgcctgaagcggctgtgtcactttcgcgcaagcaacatcaggttctgagctgcattgcgaatcaaatgacaacggaagatattctggagaaactgaaaatatcgctaaaaacgttctactgccataaacacaatatcatgatgatcctcaatcttaagcggatcaatgagctggtacgccatcagcatattgattatctggtgtga